European Patent Specification EP 4 125 999 B1, published November 6, 2024. Title: Therapeutic Agents, Pharmaceutical Compositions, and Associated Biomarkers. Applicant: Instituto de Medicina Molecular João Lobo Antunes Universidade de Coimbra Faculdade de Medicina da Universidade de Lisboa. The sequence listing filed with the application follows.

SEQUENCE LISTING (28 sequences)

SEQ ID NO: 1 - protein, 821 aa, Homo sapiens
MSPWLKWHGPAMARLWGLCLLVLGFWRASLACPTSCKCSSARIWCTEPSPGIVAFPRLEPNSVDPENITEILIANQKRLEIINEDDVEAYVGLRNLTIVDSGLKFVAYKAFLKNSNLRHINFTRNKLTSLSRRHFRHLDLSDLILTGNPFTCSCDIMWLKTLQETKSSPDTQDLYCLNESSKNMPLANLQIPNCGLPSARLAAPNLTVEEGKSVTLSCSVGGDPLPTLYWDVGNLVSKHMNETSHTQGSLRITNISSDDSGKQISCVAENLVGEDQDSVNLTVHFAPTITFLESPTSDHHWCIPFTVRGNPKPALQWFYNGAILNESKYICTKIHVTNHTEYHGCLQLDNPTHMNNGDYTLMAKNEYGKDERQISAHFMGRPGVDYETNPNYPEVLYEDWTTPTDIGDTTNKSNEIPSTDVADQSNREHLSVYAVVVIASVVGFCLLVMLLLLKLARHSKFGMKGPASVISNDDDSASPLHHISNGSNTPSSSEGGPDAVIIGMTKIPVIENPQYFGITNSQLKPDTFVQHIKRHNIVLKRELGEGAFGKVFLAECYNLCPEQDKILVAVKTLKDASDNARKDFHREAELLTNLQHEHIVKFYGVCVEGDPLIMVFEYMKHGDLNKFLRAHGPDAVLMAEGNPPTELTQSQMLHIAQQIAAGMVYLASQHFVHRDLATRNCLVGENLLVKIGDFGMSRDVYSTDYYRVGGHTMLPIRWMPPESIMYRKFTTESDVWSLGVVLWEIFTYGKQPWYQLSNNEVIECITQGRVLQRPRTCPQEVYELMLGCWQREPHTRKNIKSIHTLLQNLAKASPVYLDILG

SEQ ID NO: 2 - protein, 301 aa, Homo sapiens
SQLKPDTFVQHIKRHNIVLKRELGEGAFGKVFLAECYNLCPEQDKILVAVKTLKDASDNARKDFHREAELLTNLQHEHIVKFYGVCVEGDPLIMVFEYMKHGDLNKFLRAHGPDAVLMAEGNPPTELTQSQMLHIAQQIAAGMVYLASQHFVHRDLATRNCLVGENLLVKIGDFGMSRDVYSTDYYRVGGHTMLPIRWMPPESIMYRKFTTESDVWSLGVVLWEIFTYGKQPWYQLSNNEVIECITQGRVLQRPRTCPQEVYELMLGCWQREPHTRKNIKSIHTLLQNLAKASPVYLDILG

SEQ ID NO: 3 - protein, 520 aa, Homo sapiens
MSPWLKWHGPAMARLWGLCLLVLGFWRASLACPTSCKCSSARIWCTEPSPGIVAFPRLEPNSVDPENITEILIANQKRLEIINEDDVEAYVGLRNLTIVDSGLKFVAYKAFLKNSNLRHINFTRNKLTSLSRRHFRHLDLSDLILTGNPFTCSCDIMWLKTLQETKSSPDTQDLYCLNESSKNMPLANLQIPNCGLPSARLAAPNLTVEEGKSVTLSCSVGGDPLPTLYWDVGNLVSKHMNETSHTQGSLRITNISSDDSGKQISCVAENLVGEDQDSVNLTVHFAPTITFLESPTSDHHWCIPFTVRGNPKPALQWFYNGAILNESKYICTKIHVTNHTEYHGCLQLDNPTHMNNGDYTLMAKNEYGKDERQISAHFMGRPGVDYETNPNYPEVLYEDWTTPTDIGDTTNKSNEIPSTDVADQSNREHLSVYAVVVIASVVGFCLLVMLLLLKLARHSKFGMKGPASVISNDDDSASPLHHISNGSNTPSSSEGGPDAVIIGMTKIPVIENPQYFGITN

SEQ ID NO: 4 - protein, 4 aa, Artificial Sequence
  Artificial peptide
GITN

SEQ ID NO: 5 - protein, 5 aa, Artificial Sequence
  Artificial peptide
FGITN

SEQ ID NO: 6 - protein, 6 aa, Artificial Sequence
  Artificial peptide
YFGITN

SEQ ID NO: 7 - protein, 7 aa, Artificial Sequence
  Artificial peptide
QYFGITN

SEQ ID NO: 8 - protein, 8 aa, Artificial Sequence
  Artificial peptide
PQYFGITN

SEQ ID NO: 9 - protein, 9 aa, Artificial Sequence
  Artificial peptide
NPQYFGITN

SEQ ID NO: 10 - protein, 10 aa, Artificial Sequence
  Artificial peptide
ENPQYFGITN

SEQ ID NO: 11 - protein, 4 aa, Artificial Sequence
  Artificial peptide
SQLK

SEQ ID NO: 12 - protein, 5 aa, Artificial Sequence
  Artificial peptide
SQLKP

SEQ ID NO: 13 - protein, 6 aa, Artificial Sequence
  Artificial peptide
SQLKPD

SEQ ID NO: 14 - protein, 7 aa, Artificial Sequence
  Artificial peptide
SQLKPDT

SEQ ID NO: 15 - protein, 8 aa, Artificial Sequence
  Artificial peptide
SQLKPDTF

SEQ ID NO: 16 - protein, 9 aa, Artificial Sequence
  Artificial peptide
SQLKPDTFV

SEQ ID NO: 17 - protein, 10 aa, Artificial Sequence
  Artificial peptide
SQLKPDTFVQ

SEQ ID NO: 18 - protein, 10 aa, Artificial Sequence
  Artificial peptide
FGITNSQLKP

SEQ ID NO: 19 - protein, 16 aa, Artificial Sequence
  Artificial peptide
PQYFGITNSQLKPDTF

SEQ ID NO: 20 - protein, 14 aa, Artificial Sequence
  Artificial peptide
ITNSQLKPDTFVQH

SEQ ID NO: 21 - protein, 11 aa, Artificial Sequence
  Artificial peptide
YGRKKRRQRRR

SEQ ID NO: 22 - protein, 23 aa, Artificial Sequence
  Artificial peptide
YGRKKRRQRRRKKFGITNSQLKP

SEQ ID NO: 23 - protein, 29 aa, Artificial Sequence
  Artificial peptide
YGRKKRRQRRRKKPQYFGITNSQLKPDTF

SEQ ID NO: 24 - protein, 27 aa, Artificial Sequence
  Artificial peptide
YGRKKRRQRRRKKITNSQLKPDTFVQH

SEQ ID NO: 25 - protein, 27 aa, Artificial Sequence
  Artificial peptide
YGRKKRRQRRRPQYFGITNSQLKPDTF

SEQ ID NO: 26 - protein, 23 aa, Artificial Sequence
  Artificial peptide
YGRKKRRQRRRPPFGITNSQLKP

SEQ ID NO: 27 - protein, 22 aa, Artificial Sequence
  Artificial peptide
YGRKKRRQRRRQFGITNSQLKP

SEQ ID NO: 28 - protein, 22 aa, Artificial Sequence
  Artificial peptide
YGRKKRRQRRREFGITNSQLKP